European Patent Specification EP 3 285 788 B1, published December 18, 2024. Title: MODULATION OF AAV VECTOR TRANSGENE EXPRESSION. Applicant: University of Massachusetts. Application NOT YET ASSIGNED. The sequence listing filed with the application follows.

SEQUENCE LISTING (15 sequences)

SEQ ID NO: 1 - DNA, 260 bp, Artificial Sequence
  Synthetic Polynucleotide
ccacgttctgcttcactctccccatctcccccccctccccacccccaattttgtatttatttattttttaattattttgtgcagcgatgggggcggggggggggggcgcgcgccaggcggggcggggcggggcgaggggcggggcggggcgaggcggagaggtgcggcggcagccaatcagagcggcgcgctccgaaagtttccttttatggcgaggcggcggcggcggcggccctataaaaagcgaagcgcgcggcggg

SEQ ID NO: 2 - DNA, 110 bp, Artificial Sequence
  Synthetic Polynucleotide
tcgactctgacggttcactaaacgagctctgcttatatagcaacctgagtgatggctccgcccacgcgtgcacgtcaccgttaccggagcaacctgacaccggctccagc

SEQ ID NO: 3 - DNA, 5964 bp, Artificial Sequence
  Synthetic Polynucleotide
agcttaaaaactagcgctagcaacaacccccggaggtgcagcggctggccagagcgcccactgcctaacggagagaccccatcgtggcgcgatcatgctccgggtccccctgtgtacgccgctcccgctcctggcactgctgcaactgctgggcgctgcgcacggcatctataatgtcacccagaggacatttaagctcgactacagccgggaccgcttcctcaaggatggacagccattccgatacatctcgggaagcattcattacttccggataccccgcttctactgggaggaccggctgctgaagatgaagatggctgggctgaatgctatccagatgtacgtgccctggaacttccatgaaccccaaccaggacaatatgagttttctggggaccgtgatgtggagcatttcatccagctggctcatgagctgggactcctggtgatcctgaggcctgggccctacatctgtgcagagtgggacatggggggcttacctgcttggctactagagaaacaatctatcgttctccggtcttctgacccagactaccttgtagctgtggataaatggctggcagtccttctgcccaagatgaagcccctgctctaccagaacggaggaccgatcataaccgtgcaggttgagaatgagtacgggtcctactttgcctgcgattacgactacctacgcttcctggtgcaccgcttccgctaccatctgggtaatgacgtcattctcttcaccaccgacggagcaagtgaaaaaatgctgaagtgtgggaccctgcaggacctgtacgccacagtggattttggaacaggcaacaatatcacacaagctttcctggtccagaggaagtttgaacctaaaggacctttgatcaattctgagttctatactggctggctagaccactggggtaaaccccattccacggtgaaaactaaaacactggctacctccctctataacctgcttgcccgtggggccaacgtgaacttgtacatgtttataggtgggaccaattttgcctattggaatggtgccaacacgccctatgagccacagcccaccagctatgactacgacgccccactgagcgaggctggggacctcactaagaagtattttgctcttcgagaagtcattcagatgtttaaagaagtcccagaaggccctatccctccgtctacacccaaatttgcatatggaaaagttgctctgagaaagttcaagacagtggctgaagctctgggtatcctgtgtcccaatgggccagtgaaaagcctctatcccctgacattcactcaggtaaaacagtattttgggtatgtgctgtaccgaacaacgcttcctcaagattgcagtaacccgaaacccattttctcttcacccttcaatggtgtccgtgatcgggcttacgtctctgtggacggggtcccccaaggaatccttgatcgaaacctcatgacagctctgaacatacgggggaaggctggagccacgctggacatcctggtggagaacatggggcgtgtgaactatggcagattcatcaatgacttcaagggtttgatttccaacatgactatcaactccactgtcctcaccaactggacggtcttcccactgaacactgaggccatggtacgcaaccatctctggggccgggaggccagtgatgagggtcaccttgacggacggtcgacctccaattcttcggacctcatactccccaccttttacgtgggcaacttctccatcccctcgggcatcccagacctgccacaggacaccttcatccagtttcctgggtggtccaagggtcaagtatggatcaatggctttaacctcggccgatactggcccacaatgggcccacaaaagaccttgttcgtgccaaggaacatcctgaccacttcagccccaaacaacatcacagtgttggagctagagtttgcaccctgcagcgaggggaccccagagctgtgtacagtagagtttgttgacactccggtcatttcctgacgctagcggccgcagagatccagacatgataagatacattgatgagtttggacaaaccacaactagaatgcagtgaaaaaaatgctttatttgtgaaatttgtgatgctattgctttatttgtaaccattataagctgcaataaacaagttaacaacaacaattgcattcattttatgtttcaggttcagggggaggtgtgggaggttttttagtcgactagagctcgctgatcagcctcgactgtgccttctagttgccagccatctgttgtttgcccctcccccgtgccttccttgaccctggaaggtgccactcccactgtcctttcctaataaaatgaggaaattgcatcgcattgtctgagtaggtgtcattctattctggggggtggggtggggcaggacagcaagggggaggattgggaagacaatagcaggcatgctggggagagatctaggaacccctagtgatggagttggccactccctctctgcgcgctcgctcgctcactgaggccgcccgggcaaagcccgggcgtcgggcgacctttggtcgcccggcctcagtgagcgagcgagcgcgcagagagggagtggccatgcagccagctggcgtaatagcgaagaggcccgcaccgatcgcccttcccaacagttgcgtagcctgaatggcgaatggcgcgacgcgccctgtagcggcgcattaagcgcggcgggtgtggtggttacgcgcagcgtgaccgctacacttgccagcgccctagcgcccgctcctttcgctttcttcccttcctttctcgccacgttcgccggctttccccgtcaagctctaaatcgggggctccctttagggttccgatttagtgctttacggcacctcgaccccaaaaaacttgattagggtgatggttcacgtagtgggccatcgccctgatagacggtttttcgccctttgacgttggagtccacgttctttaatagtggactcttgttccaaactggaacaacactcaaccctatctcggtctattcttttgatttataagggattttgccgatttcggcctattggttaaaaaatgagctgatttaacaaaaatttaacgcgaattttaacaaaatattaacgtttacaatttcctgatgcggtattttctccttacgcatctgtgcggtatttcacaccgcatatggtgcactctcagtacaatctgctctgatgccgcatagttaagccagccccgacacccgccaacacccgctgacgcgccctgacgggcttgtctgctcccggcatccgcttacagacaagctgtgaccgtctccgggagctgcatgtgtcagaggttttcaccgtcatcaccgaaacgcgcgagacgaaagggcctcgtgatacgcctatttttataggttaatgtcatgataataatggtttcttagacgtcaggtggcacttttcggggaaatgtgcgcggaacccctatttgtttatttttctaaatacattcaaatatgtatccgctcatgagacaataaccctgataaatgcttcaataatattgaaaaaggaagagtatgagtattcaacatttccgtgtcgcccttattcccttttttgcggcattttgccttcctgtttttgctcacccagaaacgctggtgaaagtaaaagatgctgaagatcagttgggtgcacgagtgggttacatcgaactggatctcaacagcggtaagatccttgagagttttcgccccgaagaacgttttccaatgatgagcacttttaaagttctgctatgtggcgcggtattatcccgtattgacgccgggcaagagcaactcggtcgccgcatacactattctcagaatgacttggttgagtactcaccagtcacagaaaagcatcttacggatggcatgacagtaagagaattatgcagtgctgccataaccatgagtgataacactgcggccaacttacttctgacaacgatcggaggaccgaaggagctaaccgcttttttgcacaacatgggggatcatgtaactcgccttgatcgttgggaaccggagctgaatgaagccataccaaacgacgagcgtgacaccacgatgcctgtagcaatggcaacaacgttgcgcaaactattaactggcgaactacttactctagcttcccggcaacaattaatagactggatggaggcggataaagttgcaggaccacttctgcgctcggcccttccggctggctggtttattgctgataaatctggagccggtgagcgtgggtctcgcggtatcattgcagcactggggccagatggtaagccctcccgtatcgtagttatctacacgacggggagtcaggcaactatggatgaacgaaatagacagatcgctgagataggtgcctcactgattaagcattggtaactgtcagaccaagtttactcatatatactttagattgatttaaaacttcatttttaatttaaaaggatctaggtgaagatcctttttgataatctcatgaccaaaatcccttaacgtgagttttcgttccactgagcgtcagaccccgtagaaaagatcaaaggatcttcttgagatcctttttttctgcgcgtaatctgctgcttgcaaacaaaaaaaccaccgctaccagcggtggtttgtttgccggatcaagagctaccaactctttttccgaaggtaactggcttcagcagagcgcagataccaaatactgtccttctagtgtagccgtagttaggccaccacttcaagaactctgtagcaccgcctacatacctcgctctgctaatcctgttaccagtggctgctgccagtggcgataagtcgtgtcttaccgggttggactcaagacgatagttaccggataaggcgcagcggtcgggctgaacggggggttcgtgcacacagcccagcttggagcgaacgacctacaccgaactgagatacctacagcgtgagcattgagaaagcgccacgcttcccgaagggagaaaggcggacaggtatccggtaagcggcagggtcggaacaggagagcgcacgagggagcttccagggggaaacgcctggtatctttatagtcctgtcgggtttcgccacctctgacttgagcgtcgatttttgtgatgctcgtcaggggggcggagcctatggaaaaacgccagcaacgcggcctttttacggttcctggccttttgctggccttttgctcacatgttctttcctgcgttatcccctgattctgtggataaccgtattaccgcctttgagtgagctgataccgctcgccgcagccgaacgaccgagcgcagcgagtcagtgagcgaggaagcggaagagcgcccaatacgcaaaccgcctctccccgcgcgttggccgattcattaatgcagctgggctgcaggggggggggggggggggtggggggggggggggggggttggccactccctctctgcgcgctcgctcgctcactgaggccgggcgaccaaaggtcgcccgacgcccgggctttgcccgggcggcctcagtgagcgagcgagcgcgcagagagggagtggccaactccatcactaggggttcctagatctgaattctctagtccacgttctgcttcactctccccatctcccccccctccccacccccaattttgtatttatttattttttaattattttgtgcagcgatgggggcggggggggggggcgcgcgccaggcggggcggggcggggcgaggggcggggcggggcgaggcggagaggtgcggcggcagccaatcagagcggcgcgctccgaaagtttccttttatggcgaggcggcggcggcggcggccctataaaaagcgaagcgcgcggcggggggccgcgggccgatccaccggta

SEQ ID NO: 4 - DNA, 594 bp, Artificial Sequence
  Synthetic Polynucleotide
ccacgttctgcttcactctccccatctcccccccctccccacccccaattttgtatttatttattttttaattattttgtgcagcgatgggggcggggggggggggcgcgcgccaggcggggcggggcggggcgaggggcggggcggggcgaggcggagaggtgcggcggcagccaatcagagcggcgcgctccgaaagtttccttttatggcgaggcggcggcggcggcggccctataaaaagcgaagcgcgcggcggggggccgcggggagtcgctgcgacgctgccttcgccccgtgccccgctccgccgccgcctcgcgccgcccgccccggctctgactgaccgcgttactcccacaggtgagcgggcgggacggcccttctcctccgggctgtaattagcgcttggtttaatgacggcttgtttcttttctgtggctgcgtgaaagccttgaggggctccgggagctagagcctctgctaaccatgttcatgccttcttctttttcctacagctcctgggcaacgtgctggttattgtgctgtctcatcattttggcaaagaattcctcgaagatccgaaggggttca

SEQ ID NO: 5 - DNA, 408 bp, Artificial Sequence
  Synthetic Polynucleotide
ctggagccggtgtcaggttgctccggtaacggtgacgtgcacgcgtgggcggagccatcacgcaggttgctatataagcagagctcgtttagtgaaccgtcagaggagtcgctgcgacgctgccttcgccccgtgccccgctccgccgccgcctcgcgccgcccgccccggctctgactgaccgcgttactcccacaggtgagcgggcgggacggcccttctcctccgggctgtaattagcgcttggtttaatgacggcttgtttcttttctgtggctgcgtgaaagccttgaggggctccgggagctagagcctctgctaaccatgttcatgccttcttctttttcctacagctcctgggcaacgtgctggttattgtgctgtctcatcattttggcaaagaattcc

SEQ ID NO: 6 - DNA, 5688 bp, Artificial Sequence
  Synthetic Polynucleotide
ttggccactccctctctgcgcgctcgctcgctcactgaggccgggcgaccaaaggtcgcccgacgcccgggctttgcccgggcggcctcagtgagcgagcgagcgcgcagagagggagtggccaactccatcactaggggttcctagatctgaattcggtaccctggagccggtgtcaggttgctccggtaacggtgacgtgcacgcgtgggcggagccatcacgcaggttgctatataagcagagctcgtttagtgaaccgtcagaggagtcgctgcgacgctgccttcgccccgtgccccgctccgccgccgcctcgcgccgcccgccccggctctgactgaccgcgttactcccacaggtgagcgggcgggacggcccttctcctccgggctgtaattagcgcttggtttaatgacggcttgtttcttttctgtggctgcgtgaaagccttgaggggctccgggagctagagcctctgctaaccatgttcatgccttcttctttttcctacagctcctgggcaacgtgctggttattgtgctgtctcatcattttggcaaagaattcctcgaagatccgaaggggttcaagcttaaaaactagtggagcaccatggcaagctccaggctttggttttcgctgctgctggcggcagcgttcgcaggacgggcgaccgccctctggccctggcctcagaacatccaaacctccgaccagcgctacgtcctttatccgaacaactttcaattccagtacgatatcagctccgccgcgcagcctggctgctcagtcctcgacgaggccttccagcgctatcgtgacctgcttttcggttccgggtcttggccccgtccttaccgcacaggaaaacggcatacacctgagaagaatgtgttggttgtctctgtagtcacacctggatgtaaccagcttcctactttggagtcggtagagaattataccctgaccataaatgatgaccagtgtttactcctctctgagactgtctggggagctctccgaggtctggagacttttagccagcttgtttggaaatctgctgagggcacattctttatcaacaagactgagatcgaggactttccccgctttcctcaccggggcttgctgttggatacatctcgccattacctaccactctctagcatcctggacacactggatgtcatggcgtacaataaattgaacgtgttccactggcatctggtagatgatccttccttcccatatgagagcttcacttttccagagctcatgagaaaggggtcctacaaccctgtcacccacatttacacagcacaggatgtgaaggaggtcattgaatacgcacggctccggggtatccgtgtgcttgcagagtttgacactcctggccacactttgtcttggggaccaggtatccctggattactgactccttgctactctgggtctgagccctctggcacctttggaccagtgaatcccagtctcaacaatacctatgagttcatgagcacattcttcttggagatcagctctgtcttcccagatttttatcttcatcttggaggagatgaggttgatttcacctgctggaagtccaacccagatatccaagactttatgaggaagaaaggcttcggtgaggacttcaagcagttggagtccttctacatccagacgctgctggacatcgtctcttcttatggcaagggctatgtggtgtggcaggaggtgtttgataataaagtaaagattcggccagacacaatcatacaggtgtggcgagaagagattccagtgaactatatgaaggagctggaactggtcaccaaggccggcttccgggcccttctctccgccccctggtacctgaaccgtatatcctacggccctgactggaaggatttctacatagtggaacccctggcatttgaaggtacccctgagcagaaggctctcgtgattggtggagaggcttgtatgtggggagaatatgtggacaacacaaacctggtccccaggctctggcccagagcaggggctgttgccgaaaggctgtggagcaacaagttgacatctgacctgacatttgcctatgaacgtttgtcacacttccgctgtgagttgctgaggcgaggtgtccaggcccaacccctccatgtaggctactgtgagcaggagtttgaacagacctgactcgagctagcggccgcagagatccagacatgataagatacattgatgagtttggacaaaccacaactagaatgcagtgaaaaaaatgctttatttgtgaaatttgtgatgctattgctttatttgtaaccattataagctgcaataaacaagttaacaacaacaattgcattcattttatgtttcaggttcagggggaggtgtgggaggttttttagtcgactagagctcgctgatcagcctcgactgtgccttctagttgccagccatctgttgtttgcccctcccccgtgccttccttgaccctggaaggtgccactcccactgtcctttcctaataaaatgaggaaattgcatcgcattgtctgagtaggtgtcattctattctggggggtggggtggggcaggacagcaagggggaggattgggaagacaatagcaggcatgctggggagagatctaggaacccctagtgatggagttggccactccctctctgcgcgctcgctcgctcactgaggccgcccgggcaaagcccgggcgtcgggcgacctttggtcgcccggcctcagtgagcgagcgagcgcgcagagagggagtggccatgcagccagctggcgtaatagcgaagaggcccgcaccgatcgcccttcccaacagttgcgtagcctgaatggcgaatggcgcgacgcgccctgtagcggcgcattaagcgcggcgggtgtggtggttacgcgcagcgtgaccgctacacttgccagcgccctagcgcccgctcctttcgctttcttcccttcctttctcgccacgttcgccggctttccccgtcaagctctaaatcgggggctccctttagggttccgatttagtgctttacggcacctcgaccccaaaaaacttgattagggtgatggttcacgtagtgggccatcgccctgatagacggtttttcgccctttgacgttggagtccacgttctttaatagtggactcttgttccaaactggaacaacactcaaccctatctcggtctattcttttgatttataagggattttgccgatttcggcctattggttaaaaaatgagctgatttaacaaaaatttaacgcgaattttaacaaaatattaacgtttacaatttcctgatgcggtattttctccttacgcatctgtgcggtatttcacaccgcatatggtgcactctcagtacaatctgctctgatgccgcatagttaagccagccccgacacccgccaacacccgctgacgcgccctgacgggcttgtctgctcccggcatccgcttacagacaagctgtgaccgtctccgggagctgcatgtgtcagaggttttcaccgtcatcaccgaaacgcgcgagacgaaagggcctcgtgatacgcctatttttataggttaatgtcatgataataatggtttcttagacgtcaggtggcacttttcggggaaatgtgcgcggaacccctatttgtttatttttctaaatacattcaaatatgtatccgctcatgagacaataaccctgataaatgcttcaataatattgaaaaaggaagagtatgagtattcaacatttccgtgtcgcccttattcccttttttgcggcattttgccttcctgtttttgctcacccagaaacgctggtgaaagtaaaagatgctgaagatcagttgggtgcacgagtgggttacatcgaactggatctcaacagcggtaagatccttgagagttttcgccccgaagaacgttttccaatgatgagcacttttaaagttctgctatgtggcgcggtattatcccgtattgacgccgggcaagagcaactcggtcgccgcatacactattctcagaatgacttggttgagtactcaccagtcacagaaaagcatcttacggatggcatgacagtaagagaattatgcagtgctgccataaccatgagtgataacactgcggccaacttacttctgacaacgatcggaggaccgaaggagctaaccgcttttttgcacaacatgggggatcatgtaactcgccttgatcgttgggaaccggagctgaatgaagccataccaaacgacgagcgtgacaccacgatgcctgtagcaatggcaacaacgttgcgcaaactattaactggcgaactacttactctagcttcccggcaacaattaatagactggatggaggcggataaagttgcaggaccacttctgcgctcggcccttccggctggctggtttattgctgataaatctggagccggtgagcgtgggtctcgcggtatcattgcagcactggggccagatggtaagccctcccgtatcgtagttatctacacgacggggagtcaggcaactatggatgaacgaaatagacagatcgctgagataggtgcctcactgattaagcattggtaactgtcagaccaagtttactcatatatactttagattgatttaaaacttcatttttaatttaaaaggatctaggtgaagatcctttttgataatctcatgaccaaaatcccttaacgtgagttttcgttccactgagcgtcagaccccgtagaaaagatcaaaggatcttcttgagatcctttttttctgcgcgtaatctgctgcttgcaaacaaaaaaaccaccgctaccagcggtggtttgtttgccggatcaagagctaccaactctttttccgaaggtaactggcttcagcagagcgcagataccaaatactgtccttctagtgtagccgtagttaggccaccacttcaagaactctgtagcaccgcctacatacctcgctctgctaatcctgttaccagtggctgctgccagtggcgataagtcgtgtcttaccgggttggactcaagacgatagttaccggataaggcgcagcggtcgggctgaacggggggttcgtgcacacagcccagcttggagcgaacgacctacaccgaactgagatacctacagcgtgagcattgagaaagcgccacgcttcccgaagggagaaaggcggacaggtatccggtaagcggcagggtcggaacaggagagcgcacgagggagcttccagggggaaacgcctggtatctttatagtcctgtcgggtttcgccacctctgacttgagcgtcgatttttgtgatgctcgtcaggggggcggagcctatggaaaaacgccagcaacgcggcctttttacggttcctggccttttgctggccttttgctcacatgttctttcctgcgttatcccctgattctgtggataaccgtattaccgcctttgagtgagctgataccgctcgccgcagccgaacgaccgagcgcagcgagtcagtgagcgaggaagcggaagagcgcccaatacgcaaaccgcctctccccgcgcgttggccgattcattaatgcagctgggctgcaggggggggggggggggggtgggggggggggggggggg

SEQ ID NO: 7 - DNA, 26 bp, Artificial Sequence
  Synthetic Polynucleotide
aaacgtctcactagtccgcggaattc

SEQ ID NO: 8 - DNA, 26 bp, Artificial Sequence
  Synthetic Polynucleotide
aaacgtctcactgagaattgatcaaa

SEQ ID NO: 9 - DNA, 25 bp, Artificial Sequence
  Synthetic Polynucleotide
aaaggtctccggccgctagcgtcag

SEQ ID NO: 10 - DNA, 26 bp, Artificial Sequence
  Synthetic Polynucleotide
aaaggtctcatcagttctatactggc

SEQ ID NO: 11 - DNA, 36 bp, Artificial Sequence
  Synthetic Polynucleotide
agcatttttttcactgcattctagttgtggtttgtc

SEQ ID NO: 12 - DNA, 4260 bp, Artificial Sequence
  Synthetic Polynucleotide
ttggccactccctctctgcgcgctcgctcgctcactgaggccgggcgaccaaaggtcgcccgacgcccgggctttgcccgggcggcctcagtgagcgagcgagcgcgcagagagggagtggccaactccatcactaggggttcctagatctgaattcggtaccgagggccctgcgtatgagtgcaagtgggttttaggaccaggatgaggcggggtgggggtgcctacctgacgaccgaccccgacccactggacaagcacccaacccccattccccaaattgcgcatcccctatcagagagggggaggggaaacaggatgcggcgaggcgcgtgcgcactgccagcttcagcaccgcggacagtgccttcgcccccgcctggcggcgcgcgccaccgccgcctcagcactgaaggcgcgctgacgtcactcgccggtcccccgcaaactccccttcccggccaccttggtcgcgtccgcgccgccgccggcccagccggaccgcaccacgcgaggcgcgagataggggggcacgggcgcgaccatctgcgctgcggcgccggcgactcagcgctgcctcagtctgcggtgggcagcggaggagtcgtgtcgtgcctgagagcgcagtcgagaactagattaattaaaccggtaagcttgccaccatggtgagcaagggcgaggagctgttcaccggggtggtgcccatcctggtcgagctggacggcgacgtaaacggccacaagttcagcgtgtccggcgagggcgagggcgatgccacctacggcaagctgaccctgaagttcatctgcaccaccggcaagctgcccgtgccctggcccaccctcgtgaccaccctgacctacggcgtgcagtgcttcagccgctaccccgaccacatgaagcagcacgacttcttcaagtccgccatgcccgaaggctacgtccaggagcgcaccatcttcttcaaggacgacggcaactacaagacccgcgccgaggtgaagttcgagggcgacaccctggtgaaccgcatcgagctgaagggcatcgacttcaaggaggacggcaacatcctggggcacaagctggagtacaactacaacagccacaacgtctatatcatggccgacaagcagaagaacggcatcaaggtgaacttcaagatccgccacaacatcgaggacggcagcgtgcagctcgccgaccactaccagcagaacacccccatcggcgacggccccgtgctgctgcccgacaaccactacctgagcacccagtccgccctgagcaaagaccccaacgagaagcgcgatcacatggtcctgctggagttcgtgaccgccgccgggatcactctcggcatggacgagctgtacaagtccggactcagatcctactgaactagtcggcgacggtgctagcgtcgaccagtggatcctggaggcttgctgaaggctgtatgctgatgaacatggaatccatgcaggttttggccactgactgacctgcatggtccatgttcatcaggacacaaggcctgttactagcactcacatggaacaaatggcccagatcctggaggcttgctgaaggctgtatgctgatgaacatggaatccatgcaggttttggccactgactgacctgcatggtccatgttcatcaggacacaaggcctgttactagcactcacatggaacaaatggcccagatctggccgcactcgaaaacgggcccgcggccgcagagatccagacatgataagatacattgatgagtttggacaaaccacaactagaatgcagtgaaaaaaatgctttatttgtgaaatttgtgatgctattgctttatttgtaaccattataagctgcaataaacaagttaacaacaacaattgcattcattttatgtttcaggttcagggggaggtgtgggaggttttttagtcgacaacatatcctggtgtggagtaggggacgctgctctgacagaggctcgggggcctgagctggctctgtgagctggggaggaggcagacagccaggccttgtctgcaagcagacctggcagcattgggctggccgccccccagggcctcctcttcatgcccagtgaatgactcaccttggcacagacacaatgttcggggtgggcacagtgcctgcttcccgccgcaccccagcccccctcaaatgccttccgagaagcccattgagcagggggcttgcattgcaccccagcctgacagcctggcatcttgggataaaagcagcacagccccctaggggctgcccttgctgtgtggcgccaccggcggtggagaacaaggctctattcagcctgtgcccaggaaaggggatcaggggatgcccaggcatggacagtgggtggcagggggggagaggagggctgtctgcttcccagaagtccaaggacacaaatgggtgaggggagagctctccccatagctgggctgcggcccaaccccaccccctcaggctatgccagggggtgttgccaggggcacccgggcatcgccagtctagcccactccttcataaagccctcgcatcccaggagcgagcagagccagagcaggttggagaggagacgcatcacctccgctgctcgcttggtcgtgaggcactgggcaggtaagtatcaaggttacaagacaggtttaaggagaccaatagaaactgggcttgtcggatccacggcgacggtgctagcgtcgaccagtggatcctggaggcttgctgaaggctgtatgctgatgaacatggaatccatgcaggttttggccactgactgacctgcatggtccatgttcatcaggacacaaggcctgttactagcactcacatggaacaaatggcccagatcctggaggcttgctgaaggctgtatgctgatgaacatggaatccatgcaggttttggccactgactgacctgcatggtccatgttcatcaggacacaaggcctgttactagcactcacatggaacaaatggcccagatctggccgcactcgaaaacgggcccatcgatagagacagagaagactcttgcgtttctgataggcacctattggtcttactgacatccactttgcctttctctccacaggtgtccactcgctagcgccaccatggtgagcaagggcgaggaggataacatggccatcatcaaggagttcatgcgcttcaaggtgcacatggagggctccgtgaacggccacgagttcgagatcgagggcgagggcgagggccgcccctacgagggcacccagaccgccaagctgaaggtgaccaagggtggccccctgcccttcgcctgggacatcctgtcccctcagttcatgtacggctccaaggcctacgtgaagcaccccgccgacatccccgactacttgaagctgtccttccccgagggcttcaagtgggagcgcgtgatgaacttcgaggacggcggcgtggtgaccgtgacccaggactcctccctgcaggacggcgagttcatctacaaggtgaagctgcgcggcaccaacttcccctccgacggccccgtaatgcagaagaagaccatgggctgggaggcctcctccgagcggatgtaccccgaggacggcgccctgaagggcgagatcaagcagaggctgaagctgaaggacggcggccactacgacgctgaggtcaagaccacctacaaggccaagaagcccgtgcagctgcccggcgcctacaacgtcaacatcaagttggacatcacctcccacaacgaggactacaccatcgtggaacagtacgaacgcgccgagggccgccactccaccggcggcatggacgagctgtacaagtgacgtacggtcgactagagctcgctgatcagcctcgactgtgccttctagttgccagccatctgttgtttgcccctcccccgtgccttccttgaccctggaaggtgccactcccactgtcctttcctaataaaatgaggaaattgcatcgcattgtctgagtaggtgtcattctattctggggggtggggtggggcaggacagcaagggggaggattgggaagacaatagcaggcatgctggggagagatctaggaacccctagtgatggagttggccactccctctctgcgcgctcgctcgctcactgaggccgcccgggcaaagcccgggcgtcgggcgacctttggtcgcccggcctcagtgagcgagcgagcgcgcagagagggagtggcca

SEQ ID NO: 13 - DNA, 470 bp, Artificial Sequence
  Synthetic Polynucleotide
gagggccctgcgtatgagtgcaagtgggttttaggaccaggatgaggcggggtgggggtgcctacctgacgaccgaccccgacccactggacaagcacccaacccccattccccaaattgcgcatcccctatcagagagggggaggggaaacaggatgcggcgaggcgcgtgcgcactgccagcttcagcaccgcggacagtgccttcgcccccgcctggcggcgcgcgccaccgccgcctcagcactgaaggcgcgctgacgtcactcgccggtcccccgcaaactccccttcccggccaccttggtcgcgtccgcgccgccgccggcccagccggaccgcaccacgcgaggcgcgagataggggggcacgggcgcgaccatctgcgctgcggcgccggcgactcagcgctgcctcagtctgcggtgggcagcggaggagtcgtgtcgtgcctgagagcgcagtcgaga

SEQ ID NO: 14 - DNA, 681 bp, Artificial Sequence
  Synthetic Polynucleotide
aacatatcctggtgtggagtaggggacgctgctctgacagaggctcgggggcctgagctggctctgtgagctggggaggaggcagacagccaggccttgtctgcaagcagacctggcagcattgggctggccgccccccagggcctcctcttcatgcccagtgaatgactcaccttggcacagacacaatgttcggggtgggcacagtgcctgcttcccgccgcaccccagcccccctcaaatgccttccgagaagcccattgagcagggggcttgcattgcaccccagcctgacagcctggcatcttgggataaaagcagcacagccccctaggggctgcccttgctgtgtggcgccaccggcggtggagaacaaggctctattcagcctgtgcccaggaaaggggatcaggggatgcccaggcatggacagtgggtggcagggggggagaggagggctgtctgcttcccagaagtccaaggacacaaatgggtgaggggagagctctccccatagctgggctgcggcccaaccccaccccctcaggctatgccagggggtgttgccaggggcacccgggcatcgccagtctagcccactccttcataaagccctcgcatcccaggagcgagcagagccagagcaggttggagaggagacgcatcacctccgctgctcgc

SEQ ID NO: 15 - DNA, 45 bp, Artificial Sequence
  Synthetic Polynucleotide
caggacacaaggcctgttactagcactcacatggaacaaatggcc